European Patent Application EP 4 446 423 A1, published October 16, 2024. Title: METHOD FOR PRODUCING PROTEIN. Applicant: 味の素株式会社. The sequence listing filed with the application follows.

SEQUENCE LISTING (27 sequences)

SEQ ID NO: 1 - protein, 737 aa, Homo sapiens
MSGVFQLQLQEFINERGVLASGRPCEPGCRTFFRVCLKHFQAVVSPGPCTFGTVSTPVLGTNSFAVRDDSSGGGRNPLQLPFNFTWPGTFSLIIEAWHAPGDDLRPEALPPDALISKIAIQGSLAVGQNWLLDEQTSTLTRLRYSYRVICSDNYYGDNCSRLCKKRNDHFGHYVCQPDGNLSCLPGWTGEYCQQPICLSGCHEQNGYCSKPAECLCRPGWQGRLCNECIPHNGCRHGTCSTPWQCTCDEGWGGLFCDQDLNYCTHHSPCKNGATCSNSGQRSYTCTCRPGYTGVDCELELSECDSNPCRNGGSCKDQEDGYHCLCPPGYYGLHCEHSTLSCADSPCFNGGSCRERNQGANYACECPPNFTGSNCEKKVDRCTSNPCANGGQCLNRGPSRMCRCRPGFTGTYCELHVSDCARNPCAHGGTCHDLENGLMCTCPAGFSGRRCEVRTSIDACASSPCFNRATCYTDLSTDTFVCNCPYGFVGSRCEFPVGLPADDDDKEPKSSDKTHTCPPCPAPELLGGPSVFLFPPKPKDTLMISRTPEVTCVVVDVSHEDPEVKFNWYVDGVEVHNAKTKPREEQYNSTYRVVSVLTVLHQDWLNGKEYKCKVSNKALPAPIEKTISKAKGQPREPQVYTLPPSRDELTKNQVSLTCLVKGFYPSDIAVEWESNGQPENNYKTTPPVLDSDGSFFLYSKLTVDKSRWQQGNVFSCSVMHEALHNHYTQKSLSLSPGK

SEQ ID NO: 2 - DNA, 2214 bp, Homo sapiens
  source 1..2214: mol_type = genomic DNA
atgtctggtgttttccagctccagctgcaagagttcattaacgagaggggtgtgcttgcttctggaaggccttgtgaacctggttgcaggacttttttccgggtgtgccttaagcacttccaggctgttgtttctcctggtccttgcactttcggtactgtgtctactcctgtgctggggactaattctttcgctgtgagggatgatagcagcggtggtggtagaaatcctcttcagctgcctttcaacttcacctggcctggtacattcagcctgattattgaggcttggcacgctcctggtgatgatcttagacctgaagctttgcctcctgacgctctgatctctaagattgctatccagggttctctggctgtgggtcagaattggcttcttgatgagcagacctctaccttgaccaggctgaggtactcttacagggtgatctgcagcgataactactacggcgataactgcagccggctctgcaagaagaggaacgatcatttcggtcactacgtgtgccagcctgatggtaacctttcttgtttgcctggttggaccggtgagtattgccagcagcctatttgtctttctggttgccatgagcagaacggctactgttctaagcctgctgagtgtttgtgtaggcctggatggcagggaagattgtgcaatgagtgcattcctcacaacggttgcaggcacggtacttgttctacaccttggcagtgcacctgtgatgaaggttggggtggtcttttctgcgatcaggatcttaactactgcacccaccactctccatgcaagaatggtgctacctgctctaactctggtcagcggtcttatacttgcacttgcaggcctggttacactggtgttgattgcgagcttgagctgagcgagtgcgattctaatccttgcagaaacggtggcagctgtaaggatcaagaggatggttaccattgcttgtgccctccaggatattacggacttcattgcgagcactctaccctgtcttgtgctgattctccttgcttcaacggtggttcctgcagggaaagaaatcagggtgctaattacgcttgcgagtgccctcctaatttcaccggttctaactgcgagaagaaggtggaccgttgcacttctaacccttgcgctaatggtggtcagtgccttaatagaggccctagcagaatgtgcagatgcaggccaggattcactggaacttactgcgagctgcatgtgtctgattgcgctaggaatccttgtgctcatggtggaacttgccacgatcttgagaacggtcttatgtgcacttgccctgctggtttctctggtagaagatgcgaggtgaggacctctattgatgcttgcgcttctagcccatgcttcaatagggctacttgctacaccgatctgagcaccgatactttcgtgtgcaattgcccatacggtttcgttggttctaggtgcgagttccctgttggtttgcctgctgatgatgacgacaaagagccgaagtcctctgataagactcacacttgtcctccgtgtcctgctcctgaacttcttggtggtcctagcgttttcttgttccctccaaagcctaaggacaccctgatgatttctaggactcctgaggttacctgcgtggtggttgatgtgtctcatgaggatcccgaggtcaagttcaattggtacgttgacggtgtcgaggtgcacaacgctaagactaagcctagagaggaacagtacaacagcacctacagggttgtgtctgtgcttactgtgcttcaccaggattggctgaacggcaaagagtacaagtgtaaggtgagcaacaaggctctgcctgctcctatcgagaaaaccatctctaaggctaagggtcagcctcgtgagcctcaagtttacactttgccaccttctagggacgagctgaccaagaatcaggtgtcacttacctgcctcgtgaagggcttttacccttctgatatcgctgtcgagtgggagtctaatggacagcctgagaacaactacaagactacccctccagtgctggattccgatggttcattcttcctgtacagcaagctgaccgtggacaagtctagatggcagcagggtaatgtgttcagctgctctgttatgcatgaggcccttcacaatcactacacccagaagtccctttctctgtcccctggtaagtag

SEQ ID NO: 3 - protein, 37 aa, synthetic construct
  REGION 1..37: note = HA+His
YPYDVPDYAYPYDVPDYAYPYDVPDYAHHHHHHHHHH

SEQ ID NO: 4 - DNA, 111 bp, synthetic construct
  misc_feature 1..111: note = HA+His
  source 1..111: mol_type = other DNA
tacccttacgatgtgcctgactatgcttacccttacgatgtgcctgactatgcttacccttacgatgtgcctgactatgctcatcaccatcatcatcaccatcaccatcat

SEQ ID NO: 5 - protein, 21 aa, Arabidopsis thaliana
MAKTNLFLFLIFSLLLSLSSA

SEQ ID NO: 6 - DNA, 63 bp, Arabidopsis thaliana
  source 1..63: mol_type = genomic DNA
atggccaagaccaacctcttcctgttcctgatcttcagcctgctgctgagcctttcttctgct

SEQ ID NO: 7 - protein, 795 aa, Homo sapiens
MAAEDAAGQALQQADHTWATVVRQGLVDRAQQLLANSTALEEAMLQEQQRLGLVWAALQGARTQLRDVRAKKDQLEAHIQAAQAMLAMDTDETSKKIAHAKAVAAEAQDTATRVQSQLQAMQENVERWQGQYEGLRGQDLGQAVLDAGHSVSTLEKTLPQLLAKLSILENRGVHNASLALSASIGRVRELIAQARGAASKVKVPMKFNGRSGVQLRTPRDLADLAAYTALKFYLQGPEPEPGQGTEDRFVMYMGSRQATGDYMGVSLRDKKVHWVYQLGEAGPAVLSIDEDIGEQFAAVSLDRTLQFGHMSVTVERQMIQETKGDTVAPGAEGLLNLRPDDFVFYVGGYPSTFTPPPLLRFPGYRGCIEMDTLNEEVVSLYNFERTFQLDTAVDRPCARSKSTGDPWLTDGSYLDGTGFARISFDSQISTTKRFEQELRLVSYSGVLFFLKQQSQFLCLAVQEGSLVLLYDFGAGLKKAVPLQPPPPLTSASKAIQVFLLGGSRKRVLVRVERATVYSVEQDNDLELADAYYLGGVPPDQLPPSLRRLFPTGGSVRGCVKGIKALGKYVDLKRLNTTGVSAGCTADLLVGRAMTFHGHGFLRLALSNVAPLTGNVYSGFGFHSAQDSALLYYRASPDGLCQVSLQQGRVSLQLLRTEVKTQAGFADGAPHYVAFYSNATGVWLYVDDQLQQMKPHRGPPPELQPQPEGPPRLLLGGLPESGTIYNFSGCISNVFVQRLLGPQRVFDLQQNLGSVNVSTGCAPALQAQTPGLGPRGLQATARKASRRSRQPARHPA

SEQ ID NO: 8 - protein, 227 aa, Homo sapiens
MLQHSAADIARAEMLLEEAKRASKSATDVKVTADMVKEALEEAEKAQVAAEKAIKQADEDIQGTQNLLTSIESETAASEETLFNASQRISELERNVEELKRKAAQNSGEAEYIEKVVYTVKQSAEDVKKTLDGELDEKYKKVENLIAKKTEESADARRKAEMLQNEAKTLLAQANSKLQLLKDLERKYEDNQRYLEDKAQELARLEGEVRSLLKDISQKVAVYSTCL

SEQ ID NO: 9 - protein, 247 aa, Homo sapiens
MNDILNNLKDFDRRVNDNKTAAEEALRKIPAINQTITEANEKTREAQQALGSAAADATEAKNKAHEAERIASAVQKNATSTKAEAERTFAEVTDLDNEVNNMLKQLQEAEKELKRKQDDADQDMMMAGMASQAAQEAEINARKAKNSVTSLLSIINDLLEQLGQLDTVDLNKLNEIEGTLNKAKDEMKVSDLDRKVSDLENEAKKQEAAIMDYNRDIEEIMKDIRNLEDIRKTLPSGCFNTPSIEKP

SEQ ID NO: 10 - DNA, 2388 bp, Homo sapiens
  source 1..2388: mol_type = genomic DNA
atggctgcagaagatgctgctggtcaagcacttcaacaggctgatcatacttgggctactgttgtgaggcagggtcttgttgatagggcacaacagctgcttgctaactctaccgctcttgaagaggctatgttgcaagagcagcagaggcttggtttggtttgggctgcacttcaaggtgctagaacccagcttagagatgtgagggctaagaaggatcagcttgaggctcatattcaggctgctcaggctatgcttgctatggataccgacgagactagcaagaagatcgctcacgctaaggctgttgctgctgaagctcaagatactgctactagggtgcagtctcagctgcaagctatgcaagagaatgttgagagatggcagggacagtacgagggtcttagaggtcaggatcttggtcaggctgttcttgatgctggtcactctgtgtctaccctggaaaagactcttcctcagcttctggccaagctgagcattcttgagaataggggtgtgcacaacgcttcccttgctctgtctgcttctattggtagggtgagagagcttatcgctcaagctagaggtgctgcctctaaggttaaggtgccgatgaagttcaacggtaggtctggtgttcagcttaggactcctagagatttggctgaccttgctgcttacaccgctctgaagttttaccttcagggtcctgaacctgagcctggtcaaggtactgaggatcggttcgtgatgtatatgggtagcagacaggctaccggcgattacatgggagtttctctgagggacaagaaggtgcactgggtttaccaacttggtgaagctggtcctgctgtgctgtctatcgatgaggatattggtgagcagttcgctgctgtgtctcttgataggactcttcagttcggccacatgtctgtgactgtggaaaggcagatgatccaagagactaagggtgatactgtggctcctggtgctgagggtttgcttaatcttaggcctgacgacttcgtgttctacgttggtggttacccgtctacttttaccccacctcctttgcttaggttccctggttataggggttgcatcgagatggataccctgaacgaggaagtggtgagcctctacaatttcgagaggaccttccagcttgataccgctgttgatagaccatgcgccaggtctaagtctactggtgatccttggcttaccgacggctcttaccttgatggtactggtttcgccaggatctccttcgactctcagatttctaccaccaagcggttcgagcaagagcttaggcttgtgtcttacagcggtgtgctgttcttcctgaagcagcagtcacagttcctttgccttgctgtgcaagagggttctcttgtgctgctgtacgatttcggtgctggtctgaagaaggctgttcctcttcaacctcctccacctcttacctctgcttccaaggctattcaggtgttcctgcttggtggctctaggaagagagttctggttagagttgagcgggctaccgtgtattctgttgagcaggataacgaccttgagctggctgacgcttattaccttggtggtgttcctcctgatcagctgcctccatctcttagaaggcttttccctactggtggttctgtgaggggttgcgtgaagggtattaaggctcttggtaagtacgtggacctcaagaggcttaacactaccggtgtttctgctggctgcaccgctgatcttttggttggtagggctatgaccttccacggtcatggttttcttaggctggccctgtctaatgtggctccacttactggtaacgtgtactccggtttcggtttccactctgctcaggattctgctctgctttactacagggcttctcctgatggtctttgccaggtttcacttcagcagggtagagtgtctcttcagcttcttaggaccgaggttaagacccaggctggttttgctgatggtgctcctcattacgtggccttctactctaatgctactggcgtgtggctttacgtggacgatcaattgcaacagatgaagcctcataggggacctccacctgaattgcaacctcaacctgagggtcctccaaggcttcttcttggtggtttgcctgagtctggcaccatctacaacttcagcggctgcatctctaacgtgttcgttcagagacttctggggcctcagagggttttcgatctccaacagaatctgggcagcgtgaacgtttcaactggttgtgctcctgctctgcaagctcaaactcctggtcttggtcctagaggacttcaggctactgctaggaaggcttcaagaaggtcaagacagccagctaggcatcctgcttag

SEQ ID NO: 11 - DNA, 684 bp, Homo sapiens
  source 1..684: mol_type = genomic DNA
atgctgcaacatagcgctgctgatattgctagggctgagatgcttctggaagaggctaagagggcttctaagtctgctaccgatgttaaggtgaccgccgacatggtgaaagaggctcttgaagaagctgagaaggctcaggttgcagcagagaaggctattaagcaggccgatgaggatattcaggggacccagaatcttctgaccagcatcgaatctgagactgccgcttctgaagagactctgttcaatgcctctcagcggatctctgagcttgagaggaatgtcgaggaactgaagagaaaggctgctcagaattcaggcgaggctgagtacattgagaaggtggtgtataccgtgaagcagagcgctgaggatgtgaagaaaacccttgatggtgagctggacgagaagtacaagaaggtcgagaacctgatcgccaagaaaaccgaagagtccgctgatgctagacggaaggctgaaatgctgcagaatgaggcaaagacccttctggctcaggctaactctaagctccagctgcttaaggacttggagcggaagtacgaggataaccagagataccttgaggacaaggctcaagagcttgctaggcttgaaggtgaggtgcggtcacttctgaaggacatctctcagaaggtggccgtttactctacctgcctgtag

SEQ ID NO: 12 - DNA, 744 bp, Homo sapiens
  source 1..744: mol_type = genomic DNA
atgaacgacatcctgaacaacctgaaggacttcgacagacgggtgaacgataacaagacagctgctgaagaggccctgaggaagatccctgctattaaccagactatcaccgaggccaacgaaaagactagagaagctcaacaggctctgggttctgctgctgcagatgctactgaagctaagaacaaggctcatgaggctgagaggattgcttcagctgtgcagaagaatgccacctctactaaggctgaggcagagagaactttcgctgaggttaccgatctggacaacgaggtgaacaacatgctgaagcagcttcaagaggccgagaaagagctgaagagaaagcaggatgatgccgaccaggacatgatgatggctggtatggcttctcaggctgcacaagaagctgagatcaacgctaggaaggccaagaactctgttacctctctgctgtctatcatcaacgacctgcttgagcagcttggtcagcttgataccgtggatctcaacaagctgaacgagattgagggcaccctgaacaaggcaaaggacgagatgaaggtgagcgacctggataggaaggtgtccgatcttgagaacgaagccaagaagcaagaggctgccatcatggattacaaccgggacatcgaagagatcatgaaggacatccggaaccttgaggatatccgtaagacccttccttccggttgcttcaacaccccttctatcgagaagccgtag

SEQ ID NO: 13 - protein, 237 aa, Aequorea victoria
MATALTEGAKLFEKEIPYITELEGDVEGMKFIIKGEGTGDATTGTIKAKYICTTGDLPVPWATLVSTLSYGVQCFAKYPSHIKDFFKSAMPEGYTQERTISFEGDGVYKTRAMVTYERGSIYNRVTLTGENFKKDGHILRKNVAFQCPPSILYILPDTVNNGIRVEFNQAYDIEGVTEKLVTKCSQMNRPLAGSAAVHIPRYHHITYHTKLSKDRDERRDHMCLVEVVKAVDLDTYQ

SEQ ID NO: 14 - DNA, 714 bp, Aequorea victoria
  source 1..714: mol_type = genomic DNA
atggctactgctcttactgaaggagctaagttgtttgagaaggaaattccatatattactgaacttgagggagatgttgagggtatgaagttcattattaagggagagggaactggagatgctactacaggaactattaaggctaagtacatttgcactacaggtgatttgccagttccttgggctactcttgtttctactctttcttacggagttcagtgcttcgctaagtatccatctcatattaaggatttctttaagtctgctatgccagagggatatactcaagagaggactatttctttcgaaggagatggagtttacaagactagggctatggttacttatgagagaggatcaatttataatagagttactttgactggagagaatttcaagaaagatggacatattcttaggaagaatgttgctttccaatgtccaccttctattctttacattcttccagatactgttaataatggtattagagttgagttcaatcaagcatacgatattgaaggagttactgagaagttggttactaagtgctctcaaatgaataggccacttgctggatctgctgctgttcatattcctagataccatcatattacatatcatactaagttgtctaaggatagggatgagaggagagatcacatgtgccttgttgaggttgttaaggctgttgatcttgatacttaccaatga

SEQ ID NO: 15 - protein, 12 aa, synthetic construct
  REGION 1..12: note = YPYD+FLAG
YPYDDYKDDDDK

SEQ ID NO: 16 - DNA, 36 bp, synthetic construct
  misc_feature 1..36: note = YPYD+FLAG
  source 1..36: mol_type = other DNA
tacccttacgacgactacaaggacgacgatgacaaa

SEQ ID NO: 17 - protein, 9 aa, influenzavirus
YPYDVPDYA

SEQ ID NO: 18 - protein, 7 aa, influenzavirus
YPYDVPD

SEQ ID NO: 19 - protein, 4 aa, influenzavirus
YPYD

SEQ ID NO: 20 - DNA, 822 bp, Homo sapiens
  source 1..822: mol_type = genomic DNA
atggaagctgccccgtccaggttcatgttcctcttatttctcctcacgtgtgagctggctgcagaagttgctgcagaagttgagaaatcctcagatggtcctggtgctgcccaggaacccacgtggctcacagatgtcccagctgccatggaattcattgctgccactgaggtggctgtcataggcttcttccaggatttagaaataccagcagtgcccatactccatagcatggtgcaaaaattcccaggcgtgtcatttgggatcagcactgattctgaggttctgacacactacaacatcactgggaacaccatctgcctctttcgcctggtagacaatgaacaactgaatttagaggacgaagacattgaaagcattgatgccaccaaattgagccgtttcattgagatcaacagcctccacatggtgacagagtacaaccctgtgactgtgattgggttattcaacagcgtaattcagattcatctcctcctgataatgaacaaggcctccccagagtatgaagagaacatgcacagataccagaaggcagccaagctcttccaggggaagattctctttattctggtggacagtggtatgaaagaaaatgggaaggtgatatcatttttcaaactaaaggagtctcaactgccagctttggcaatttaccagactctagatgacgagtgggatacactgcccacagcagaagtttccgtagagcatgtgcaaaacttttgtgatggattcctaagtggaaaattgttgaaagaaaatcgtgaatcagaaggaaagactccaaaggtggaactctga

SEQ ID NO: 21 - protein, 273 aa, Homo sapiens
MEAAPSRFMFLLFLLTCELAAEVAAEVEKSSDGPGAAQEPTWLTDVPAAMEFIAATEVAVIGFFQDLEIPAVPILHSMVQKFPGVSFGISTDSEVLTHYNITGNTICLFRLVDNEQLNLEDEDIESIDATKLSRFIEINSLHMVTEYNPVTVIGLFNSVIQIHLLLIMNKASPEYEENMHRYQKAAKLFQGKILFILVDSGMKENGKVISFFKLKESQLPALAIYQTLDDEWDTLPTAEVSVEHVQNFCDGFLSGKLLKENRESEGKTPKVEL

SEQ ID NO: 22 - DNA, 843 bp, Homo sapiens
  source 1..843: mol_type = genomic DNA
atggcgccctccgggagtcttgcagttcccctggcagtcctggtgctgttgctttggggtgctccctggacgcacgggcggcggagcaacgttcgcgtcatcacggacgagaactggagagaactgctggaaggagactggatgatagaattttatgccccgtggtgccctgcttgtcaaaatcttcaaccggaatgggaaagttttgctgaatggggagaagatcttgaggttaatattgcgaaagtagatgtcacagagcagccaggactgagtggacggtttatcataactgctcttcctactatttatcattgtaaagatggtgaatttaggcgctatcagggtccaaggactaagaaggacttcataaactttataagtgataaagagtggaagagtattgagcccgtttcatcatggtttggtccaggttctgttctgatgagtagtatgtcagcactctttcagctatctatgtggatcaggacttgccataactactttattgaagaccttggattgccagtgtggggatcatatactgtttttgctttagcaactctgttttccggactgttattaggactctgtatgatatttgtggcagattgcctttgtccttcaaaaaggcgcagaccacagccgtacccatacccttcaaaaaaattattatcagaatctgcacaacctttgaaaaaagtggaggaggaacaagaggcggatgaagaagatgtttcagaagaagaagctgaaagtaaagaaggaacaaacaaagactttccacagaatgccataagacaacgctctctgggtccatcattggccacagataaatcctag

SEQ ID NO: 23 - protein, 280 aa, Homo sapiens
MAPSGSLAVPLAVLVLLLWGAPWTHGRRSNVRVITDENWRELLEGDWMIEFYAPWCPACQNLQPEWESFAEWGEDLEVNIAKVDVTEQPGLSGRFIITALPTIYHCKDGEFRRYQGPRTKKDFINFISDKEWKSIEPVSSWFGPGSVLMSSMSALFQLSMWIRTCHNYFIEDLGLPVWGSYTVFALATLFSGLLLGLCMIFVADCLCPSKRRRPQPYPYPSKKLLSESAQPLKKVEEEQEADEEDVSEEEAESKEGTNKDFPQNAIRQRSLGPSLATDKS

SEQ ID NO: 24 - DNA, 1089 bp, Homo sapiens
  source 1..1089: mol_type = genomic DNA
ggctcctgggacccggccggttacctgctctactgcccctgcatggggcgctttgggaaccaggccgatcacttcttgggctctctggcatttgcaaagctgctaaaccgtaccttggctgtccctccttggattgagtaccagcatcacaagcctcctttcaccaacctccatgtgtcctaccagaagtacttcaagctggagcccctccaggcttaccatcgggtcatcagcttggaggatttcatggagaagctggcacccacccactggccccctgagaagcgggtggcatactgctttgaggtggcagcccagcgaagcccagataagaagacgtgccccatgaaggaaggaaacccctttggcccattctgggatcagtttcatgtgagtttcaacaagtcggagctttttacaggcatttccttcagtgcttcctacagagaacaatggagccagagattttctccaaaggaacatccggtgcttgccctgccaggagccccagcccagttccccgtcctagaggaacacaggccactacagaagtacatggtatggtcagacgaaatggtgaagacgggagaggcccagattcatgcccaccttgtccggccctatgtgggcattcatctgcgcattggctctgactggaagaacgcctgtgccatgctgaaggacgggactgcaggctcgcacttcatggcctctccgcagtgtgtgggctacagccgcagcacagcggcccccctcacgatgactatgtgcctgcctgacctgaaggagatccagagggctgtgaagctctgggtgaggtcgctggatgcccagtcggtctacgttgctactgattccgagagttatgtgcctgagctccaacagctcttcaaagggaaggtgaaggtggtgagcctgaagcctgaggtggcccaggtcgacctgtacatcctcggccaagccgaccactttattggcaactgtgtctcctccttcactgcctttgtgaagcgggagcgggacctccaggggaggccgtcttctttcttcggcatggacaggccccctaagctgcgggacgagttctga

SEQ ID NO: 25 - protein, 362 aa, Homo sapiens
GSWDPAGYLLYCPCMGRFGNQADHFLGSLAFAKLLNRTLAVPPWIEYQHHKPPFTNLHVSYQKYFKLEPLQAYHRVISLEDFMEKLAPTHWPPEKRVAYCFEVAAQRSPDKKTCPMKEGNPFGPFWDQFHVSFNKSELFTGISFSASYREQWSQRFSPKEHPVLALPGAPAQFPVLEEHRPLQKYMVWSDEMVKTGEAQIHAHLVRPYVGIHLRIGSDWKNACAMLKDGTAGSHFMASPQCVGYSRSTAAPLTMTMCLPDLKEIQRAVKLWVRSLDAQSVYVATDSESYVPELQQLFKGKVKVVSLKPEVAQVDLYILGQADHFIGNCVSSFTAFVKRERDLQGRPSSFFGMDRPPKLRDEF

SEQ ID NO: 26 - protein, 757 aa, Homo sapiens
MAKTNLFLFLIFSLLLSLSSASGVFQLQLQEFINERGVLASGRPCEPGCRTFFRVCLKHFQAVVSPGPCTFGTVSTPVLGTNSFAVRDDSSGGGRNPLQLPFNFTWPGTFSLIIEAWHAPGDDLRPEALPPDALISKIAIQGSLAVGQNWLLDEQTSTLTRLRYSYRVICSDNYYGDNCSRLCKKRNDHFGHYVCQPDGNLSCLPGWTGEYCQQPICLSGCHEQNGYCSKPAECLCRPGWQGRLCNECIPHNGCRHGTCSTPWQCTCDEGWGGLFCDQDLNYCTHHSPCKNGATCSNSGQRSYTCTCRPGYTGVDCELELSECDSNPCRNGGSCKDQEDGYHCLCPPGYYGLHCEHSTLSCADSPCFNGGSCRERNQGANYACECPPNFTGSNCEKKVDRCTSNPCANGGQCLNRGPSRMCRCRPGFTGTYCELHVSDCARNPCAHGGTCHDLENGLMCTCPAGFSGRRCEVRTSIDACASSPCFNRATCYTDLSTDTFVCNCPYGFVGSRCEFPVGLPADDDDKEPKSSDKTHTCPPCPAPELLGGPSVFLFPPKPKDTLMISRTPEVTCVVVDVSHEDPEVKFNWYVDGVEVHNAKTKPREEQYNSTYRVVSVLTVLHQDWLNGKEYKCKVSNKALPAPIEKTISKAKGQPREPQVYTLPPSRDELTKNQVSLTCLVKGFYPSDIAVEWESNGQPENNYKTTPPVLDSDGSFFLYSKLTVDKSRWQQGNVFSCSVMHEALHNHYTQKSLSLSPGK

SEQ ID NO: 27 - protein, 395 aa, Homo sapiens
MAKTNLFLFLIFSLLLSLSSAYPYDDYKDDDDKGSWDPAGYLLYCPCMGRFGNQADHFLGSLAFAKLLNRTLAVPPWIEYQHHKPPFTNLHVSYQKYFKLEPLQAYHRVISLEDFMEKLAPTHWPPEKRVAYCFEVAAQRSPDKKTCPMKEGNPFGPFWDQFHVSFNKSELFTGISFSASYREQWSQRFSPKEHPVLALPGAPAQFPVLEEHRPLQKYMVWSDEMVKTGEAQIHAHLVRPYVGIHLRIGSDWKNACAMLKDGTAGSHFMASPQCVGYSRSTAAPLTMTMCLPDLKEIQRAVKLWVRSLDAQSVYVATDSESYVPELQQLFKGKVKVVSLKPEVAQVDLYILGQADHFIGNCVSSFTAFVKRERDLQGRPSSFFGMDRPPKLRDEF